European Patent Specification EP 3 530 260 B1, published November 1, 2023. Title: Method for inhibiting oxidation of antioxidant using aptamer, the material and use of the same. Applicant: NEXMOS CO.,LTD. The sequence listing filed with the application follows.

SEQUENCE LISTING (2 sequences)

SEQ ID NO: 1 - DNA, 32 bp, Artificial Sequence
  Aptamer
agagctcgcgccggagttctcaatgcaagagc

SEQ ID NO: 2 - DNA, 32 bp, Artificial Sequence
  Aptamer
gtggaggcggtggccagtctcatacgcggcag